European Patent Specification EP 3 835 415 B1, published September 25, 2024. Title: A method of producing CD3-positive cells. Applicant: KYOTO UNIVERSITY TAKEDA PHARMACEUTICAL COMPANY LIMITED. The sequence listing filed with the application follows.

SEQUENCE LISTING (24 sequences)

SEQ ID NO: 1 - protein, 9 aa, Homo sapiens
RMFPNAPYL

SEQ ID NO: 2 - protein, 9 aa, Homo sapiens
SLGEQQYSV

SEQ ID NO: 3 - protein, 9 aa, Homo sapiens
CMTWNQMNL

SEQ ID NO: 4 - protein, 9 aa, Homo sapiens
CYTWNQMNL

SEQ ID NO: 5 - protein, 544 aa, Artificial Sequence
  CD19-CAR
MDWTWRILFLVAAATGAHSDIQMTQTTSSLSASLGDRVTISCRASQDISKYLNWYQQKPDGTVKLLIYHTSRLHSGVPSRFSGSGSGTDYSLTISNLEQEDIATYFCQQGNTLPYTFGGGTKLEITGGGGSGGGGSGGGGSEVKLQESGPGLVAPSQSLSVTCTVSGVSLPDYGVSWIRQPPRKGLEWLGVIWGSETTYYNSALKSRLTIIKDNSKSQVFLKMNSLQTDDTAIYYCAKHYYYGGSYAMDYWGQGTSVTVSSFVPVFLPAKPTTTPAPRPPTPAPTIASQPLSLRPEACRPAAGGAVHTRGLDFACDIYIWAPLAGTCGVLLLSLVITLYCNHRNRSKRSRLLHSDYMNMTPRRPGPTRKHYQPYAPPRDFAAYRSRFSVVKRGRKKLLYIFKQPFMRPVQTTQEEDGCSCRFPEEEEGGCELRVKFSRSADAPAYQQGQNQLYNELNLGRREEYDVLDKRRGRDPEMGGKPRRKNPQEGLYNELQKDKMAEAYSEIGMKGERRRGKGHDGLYQGLSTATKDTYDALHMQALPPR

SEQ ID NO: 6 - protein, 87 aa, Homo sapiens
HTNNKIEKIYIMKADTVIVGTVKAELPEGRGLAGPAEPELEEELEADHTPHYPEQETEPPLGSCSDVMLSVEEEGKEDPLPTAASGK

SEQ ID NO: 7 - protein, 965 aa, Artificial Sequence
  CD19-CAR(CD8-CD28-CD30-CD3z)
MDWTWRILFLVAAATGAHSDIQMTQTTSSLSASLGDRVTISCRASQDISKYLNWYQQKPDGTVKLLIYHTSRLHSGVPSRFSGSGSGTDYSLTISNLEQEDIATYFCQQGNTLPYTFGGGTKLEITGGGGSGGGGSGGGGSEVKLQESGPGLVAPSQSLSVTCTVSGVSLPDYGVSWIRQPPRKGLEWLGVIWGSETTYYNSALKSRLTIIKDNSKSQVFLKMNSLQTDDTAIYYCAKHYYYGGSYAMDYWGQGTSVTVSSFVPVFLPAKPTTTPAPRPPTPAPTIASQPLSLRPEACRPAAGGAVHTRGLDFACDIYIWAPLAGTCGVLLLSLVITLYCNHRNRSKRSRLLHSDYMNMTPRRPGPTRKHYQPYAPPRDFAAYRSHTNNKIEKIYIMKADTVIVGTVKAELPEGRGLAGPAEPELEEELEADHTPHYPEQETEPPLGSCSDVMLSVEEEGKEDPLPTAASGKRVKFSRSADAPAYQQGQNQLYNELNLGRREEYDVLDKRRGRDPEMGGKPRRKNPQEGLYNELQKDKMAEAYSEIGMKGERRRGKGHDGLYQGLSTATKDTYDALHMQALPPRLEGGGEGRGSLLTCGDVEENPGPRMLLLVTSLLLCELPHPAFLLIPRKVCNGIGIGEFKDSLSINATNIKHFKNCTSISGDLHILPVAFRGDSFTHTPPLDPQELDILKTVKEITGFLLIQAWPENRTDLHAFENLEIIRGRTKQHGQFSLAVVSLNITSLGLRSLKEISDGDVIISGNKNLCYANTINWKKLFGTSGQKTKIISNRGENSCKATGQVCHALCSPEGCWGPEPRDCVSCRNVSRGRECVDKCNLLEGEPREFVENSECIQCHPECLPQAMNITCTGRGPDNCIQCAHYIDGPHCVKTCPAGVMGENNTLVWKYADAGHVCHLCHPNCTYGCTGPGLEGCPTNGPKIPSIATGMVGALLLLLVVALGIGLFM

SEQ ID NO: 8 - protein, 400 aa, Homo sapiens
MYRMQLLSCIALSLALVTNSATSNWVNVISDLKKIEDLIQSMHIDATLYTESDVHPSCKVTAMKCFLLELQVISLESGDASIHDTVENLIILANNSLSSNGNVTESGCKECEELEEKNIKEFLQSFVHIVQMFINTSSGGGSGGGGSGGGGSGGGGSGGGSLQITCPPPMSVEHADIWVKSYSLYSRERYICNSGFKRKAGTSSLTECVLNKATNVAHWTTPSLKCIRDPALVHQRPAPPSTVTTAGVTPQPESLSPSGKEPAASSPSSNNTAATTAAIVPGSQLMPSKSPSTGTTEISSHESSHGTPSQTTAKNWELTASASHQPPGVYPQGHSDTTVAISTSTVLLCGLSAVSLLACYLKSRQTPPLASVEMEAMEALPVTWGTSSRDEDLENCSHHL

SEQ ID NO: 9 - protein, 5 aa, Mus musculus
RYTMH

SEQ ID NO: 10 - protein, 17 aa, Mus musculus
YINPSRGYTNYNQKFKD

SEQ ID NO: 11 - protein, 10 aa, Mus musculus
YYDDHYCLDY

SEQ ID NO: 12 - protein, 10 aa, Mus musculus
SASSSVSYMN

SEQ ID NO: 13 - protein, 7 aa, Mus musculus
DTSKLAS

SEQ ID NO: 14 - protein, 9 aa, Mus musculus
QQWSSNPFT

SEQ ID NO: 15 - protein, 10 aa, Mus musculus
GYSFTGYTMN

SEQ ID NO: 16 - protein, 10 aa, Mus musculus
LINPYKGVST

SEQ ID NO: 17 - protein, 13 aa, Mus musculus
SGYYGDSDWYFDV

SEQ ID NO: 18 - protein, 11 aa, Mus musculus
RASQDIRNYLN

SEQ ID NO: 19 - protein, 7 aa, Mus musculus
YTSRLHS

SEQ ID NO: 20 - protein, 9 aa, Mus musculus
QQGNTLPWT

SEQ ID NO: 21 - protein, 119 aa, Mus musculus
QVQLQESGAELARPGASVKMSCKASGYTFTRYTMHWVKQRPGQGLEWIGYINPSRGYTNYNQKFKDKATLTTDKSSSTAYMQLSSLTSEDSAVYYCARYYDDHYCLDYWGQGTTLTVSS

SEQ ID NO: 22 - protein, 107 aa, Mus musculus
QIVLTQSPAIMSASPGEKVTMTCSASSSVSYMNWYQQKSGTSPKRWIYDTSKLASGVPAHFRGSGSGTSYSLTISGMEAEDAATYYCQQWSSNPFTFGSGTKLEINR

SEQ ID NO: 23 - protein, 122 aa, Mus musculus
EVQLQQSGPELVKPGASMKISCKASGYSFTGYTMNWVKQSHGKNLEWMGLINPYKGVSTYNQKFKDKATLTVDKSSSTAYMELLSLTSEDSAVYYCARSGYYGDSDWYFDVWGAGTTVTVSS

SEQ ID NO: 24 - protein, 109 aa, Mus musculus
DIQMTQTTSSLSASLGDRVTISCRASQDIRNYLNWYQQKPDGTVKLLIYYTSRLHSGVPSKFSGSGSGTDYSLTISNLEQEDIATYFCQQGNTLPWTFAGGTKLEIKRA